European Patent Application EP 4 563 702 A1, published June 4, 2025. Title: Variant Protease. Applicant: Kao Corporation. The sequence listing filed with the application follows.

SEQUENCE LISTING (1 sequence)

SEQ ID NO: 1 - protein, 434 aa, Bacillus sp.
NDVARGIVKADVAQSVYGLYGQGQIVAVADTGLDTGRNDSSMHEAFRGKITALYALGRTNNANDPNGHGTHVAGSVLGNGSEAKGMAPQANLVFQSIMDSGGGLGGLPSNLQTLFSQAYSAGARIHTNSWGTAVNGAYTTDSRNVDDYVRKNDMTILFAAGNEGPGVGTISAPGTAKNAITVGATENLRPSFGSQADNINDVAQFSSRGPTKDGRIKPDVMAPGTFILSARSSLAPDSSFWANHDSKYAYMGGTSMATPIVAGNVAQLREHFIKNRGITPKPSLLKAALIAGATDIGLGYPNEAQGWGRVTLDKSLNVAYVNESSSLSTSQKATYSFTATAGKPLKISLVWSDAPASTSASVTLVNDLNLVITAPNGTQYVGNDFTAPYNDNWDGRNNVENVFINAPQSGTYTIEVQAYNVPVGPQTFSLAIVN